European Patent Specification EP 3 644 720 B1, published February 7, 2024. Title: NON-HUMAN MODEL FOR NEUROFIBROMATOSIS TYPE 1. Applicant: PARIS SCIENCES ET LETTRES - QUARTIER LATIN CENTRE NATIONAL DE LA RECHERCHE SCIENTIFIQUE INSTITUT NATIONAL DE LA SANTÉ ET DE LA RECHERCHE MÉDICALE TOPILKO Piotr CHARNAY Patrick COULPIER Fanny GRESSET Aurélie RADOMSKA Katarzyna. The sequence listing filed with the application follows.

SEQUENCE LISTING (18 sequences)

SEQ ID NO: 1 - DNA, 20 bp, Artificial Sequence
  Prss56 primer (Forward)
gtcacaatccccgagaacag

SEQ ID NO: 2 - DNA, 20 bp, Artificial Sequence
  Prss56 primer (Reverse)
ctcgctgaatagccgctaac

SEQ ID NO: 3 - DNA, 20 bp, Artificial Sequence
  Prss56 primer (Forward)
ggtcttcagtggcctagtgg

SEQ ID NO: 4 - DNA, 20 bp, Artificial Sequence
  Prss56 primer (Reverse)
agcctctgtccttgatcagc

SEQ ID NO: 5 - DNA, 20 bp, Artificial Sequence
  Prss56 primer (Forward)
cctagcgctccaacagtgtc

SEQ ID NO: 6 - DNA, 20 bp, Artificial Sequence
  Prss56 primer (Reverse)
agtgctcagctgggatctgt

SEQ ID NO: 7 - DNA, 20 bp, Artificial Sequence
  Prss56 primer (Forward)
atgacctggccttggtacag

SEQ ID NO: 8 - DNA, 20 bp, Artificial Sequence
  Prss56 primer (Reverse)
gacaggtgtctgcactgagc

SEQ ID NO: 9 - protein, 343 aa, Enterobacteria phage P1
  Cre recombinase
MSNLLTVHQNLPALPVDATSDEVRKNLMDMFRDRQAFSEHTWKMLLSVCRSWAAWCKLNNRKWFPAEPEDVRDYLLYLQARGLAVKTIQQHLGQLNMLHRRSGLPRPSDSNAVSLVMRRIRKENVDAGERAKQALAFERTDFDQVRSLMENSDRCQDIRNLAFLGIAYNTLLRIAEIARIRVKDISRTDGGRMLIHIGRTKTLVSTAGVEKALSLGVTKLVERWISVSGVADDPNNYLFCRVRKNGVAAPSATSQLSTRALEGIFEATHRLIYGAKDDSGQRYLAWSGHSARVGAARDMARAGVSIPEIMQAGGWTNVNIVMNYIRNLDSETGAMVRLLEDGD

SEQ ID NO: 10 - DNA, 1053 bp, Artificial Sequence
  Cre recombinase (cDNA)
atgcccaagaagaagaggaaggtgtccaatttactgaccgtacaccaaaatttgcctgcattaccggtcgatgcaacgagtgatgaggttcgcaagaacctgatggacatgttcagggatcgccaggcgttttctgagcatacctggaaaatgcttctgtccgtttgccggtcgtgggcggcatggtgcaagttgaataaccggaaatggtttcccgcagaacctgaagatgttcgcgattatcttctatatcttcaggcgcgcggtctggcagtaaaaactatccagcaacatttgggccagctaaacatgcttcatcgtcggtccgggctgccacgaccaagtgacagcaatgctgtttcactggttatgcggcggatccgaaaagaaaacgttgatgccggtgaacgtgcaaaacaggctctagcgttcgaacgcactgatttcgaccaggttcgttcactcatggaaaatagcgatcgctgccaggatatacgtaatctggcatttctggggattgcttataacaccctgttacgtatagccgaaattgccaggatcagggttaaagatatctcacgtactgacggtgggagaatgttaatccatattggcagaacgaaaacgctggttagcaccgcaggtgtagagaaggcacttagcctggaggtaactaaactggtcgagcgatggatttccgtctctggtgtagctgatgatccgaataactacctgttttgccgggtcagaaaaaatggtgttgccgcgccatctgccaccagccagctatcaactcgcgccctggaagggatttttgaagcaactcatcgattgatttacggcgctaaggatgactctggtcagagatacctggcctggtctggacacagtgcccgtgtcggagccgcgcgagatatggcccgcgctggagtttcaataccggagatcatgcaagctggtggctggaccaatgtaaatattgtcatgaactatatccgtaacctggatagtgaaacaggggcaatggtgcgcctgctggaagatggcgattag

SEQ ID NO: 11 - DNA, 34 bp, Enterobacteria phage P1
  loxP
  variation 14: /note="n is any of A, C, G or T"
  variation 15: /note="n is any of A, C, G or T"
  variation 16: /note="n is any of A, C, G or T"
  variation 19: /note="n is any of A, C, G or T"
  variation 20: /note="n is any of A, C, G or T"
  variation 21: /note="n is any of A, C, G or T"
ataacttcgtatannntannntatacgaagttat

SEQ ID NO: 12 - DNA, 34 bp, Enterobacteria phage P1
  loxP
ataacttcgtataatgtatgctatacgaagttat

SEQ ID NO: 13 - DNA, 20 bp, Artificial Sequence
  Prss56Cre knock-in primer (Forward)
caggtgaggtgcggaccatt

SEQ ID NO: 14 - DNA, 25 bp, Artificial Sequence
  Prss56Cre knock-in primer (Reverse)
acggaaatccatcgctcgaccagtt

SEQ ID NO: 15 - DNA, 20 bp, Artificial Sequence
  Beta-actin primer (forward)
tgttaccaactgggacgaca

SEQ ID NO: 16 - DNA, 20 bp, Artificial Sequence
  Beta-actin primer (reverse)
ggggtgttgaaggtctcaaa

SEQ ID NO: 17 - DNA, 20 bp, Artificial Sequence
  Nf1 primer (forward)
gcttccctcagaacagcatc

SEQ ID NO: 18 - DNA, 21 bp, Artificial Sequence
  Nf1 primer (reverse)
gcccctttcaattctaggtgg